European Patent Specification EP 3 629 719 B1, published August 23, 2023. Title: METHODS FOR GENDER DETERMINATION OF AVIAN EMBRYOS IN UNHATCHED EGGS AND MEANS THEREOF. Applicant: EGGXYT LTD. The sequence listing filed with the application follows.

SEQUENCE LISTING (67 sequences)

SEQ ID NO: 1 - DNA, 20 bp, Artificial Sequence
  Guide 1 for W chromosome
gcactaggaaccagcagcag

SEQ ID NO: 2 - DNA, 20 bp, Artificial Sequence
  Guide 2 for W chromosome
gtagccccaagagggctagg

SEQ ID NO: 3 - DNA, 1460 bp, Artificial Sequence
  galGal5_dna range=chrW:1022859-1024215
tcgggctaacattagacccgttgtgtcttaatcctgccgtcgggtatacatatactaaaagaacctcctttccctcctataaatcggagcgagacaaggcattctttttttattattattttggttgcctgcccatcagatgtaatgaaagttgcacagggtagggctaagaaggtaaaggagttaaattcccccgggaggttagagattccctgtattgtggttgcctgcccattagacgtaacaaaagttgtgaagggtaggactaaggatccaggtaaagaggttagtcccccagggttagagtccctcctcagaagtaaatgtaaaacataaccacggtaattgtcgttgagtgcgcttgtttgattgttaattgtttgtgctgttattgtatgctgattgtttgtgttgttattatacaaagagctcacatgcatcgttaaaatgggcattggatcacctaggggtgagggaattttgaaaaagtcacttttgggctgtgttttaagtcattggaaagaaatagctggatcccctggtggggttgcacagaaggatgatttaagtacgatggatgcctttgaggcaggcactaggaaccagcagcagtggcagatttgtgatcatggaaagaattggtgggagcatacggcaccaggactcagataagatagctagctaaggtgatgaattgtagatggtgtcagataacgaaagaagaaaaacaaatgtaataaagtgttaaatgccaatatgttttttataatgaggcaatatcctgaatggcattagtgtgggatcaatttggcccagatgaccctctgattttaatggtagaaaatgataagagagagagggagaaaggaagagagtgtaaaacgtgttgttcagcatgtagtattggactgagatgcttcaagcgaaacaagaatgagcaggaggaggatttagagatgctagtagccccaagagggctagggggcctcaaaatcatggaacccaactccctggagtagaagggtcaggtaatgagtccaaaagagggactataggaaccatgccagtaacagagaggactcacagccagcatagggtcgtgctgtaagccctgttgaggcagttggaaatgacagttcggtagtagttaaggtacccttttaaattacagatttaaacatttggaaagcagctgctggcagctaccgtgatgatcctaaacgggtagctaatgcttttgaaatgatgattaaaactcaggaactggataggaaagatatggaatttattatgcacatgttgtttgatagtacagaaaaataaatgattcactagaccacacggacccaagtggaggatcaggtaatggcaggggttttgcttggatgtaatgctggaaaggacaagagtcctttcctgtcctggggaggatttagaggtggttagaccttggggaggag

SEQ ID NO: 4 - DNA, 592 bp, Artificial Sequence
  For cloning using the gRNA1, W chromosome, "Left arm"
tcgggctaacattagacccgttgtgtcttaatcctgccgtcgggtatacatatactaaaagaacctcctttccctcctataaatcggagcgagacaaggcattctttttttattattattttggttgcctgcccatcagatgtaatgaaagttgcacagggtagggctaagaaggtaaaggagttaaattcccccgggaggttagagattccctgtattgtggttgcctgcccattagacgtaacaaaagttgtgaagggtaggactaaggatccaggtaaagaggttagtcccccagggttagagtccctcctcagaagtaaatgtaaaacataaccacggtaattgtcgttgagtgcgcttgtttgattgttaattgtttgtgctgttattgtatgctgattgtttgtgttgttattatacaaagagctcacatgcatcgttaaaatgggcattggatcacctaggggtgagggaattttgaaaaagtcacttttgggctgtgttttaagtcattggaaagaaatagctggatcccctggtggggttgcacagaaggatgatttaagtacgatggatgcctttgaggcag

SEQ ID NO: 5 - DNA, 848 bp, Artificial Sequence
  For cloning using the gRNA1, W chromosome, "Right arm"
tggcagatttgtgatcatggaaagaattggtgggagcatacggcaccaggactcagataagatagctagctaaggtgatgaattgtagatggtgtcagataacgaaagaagaaaaacaaatgtaataaagtgttaaatgccaatatgttttttataatgaggcaatatcctgaatggcattagtgtgggatcaatttggcccagatgaccctctgattttaatggtagaaaatgataagagagagagggagaaaggaagagagtgtaaaacgtgttgttcagcatgtagtattggactgagatgcttcaagcgaaacaagaatgagcaggaggaggatttagagatgctagtagccccaagagggctagggggcctcaaaatcatggaacccaactccctggagtagaagggtcaggtaatgagtccaaaagagggactataggaaccatgccagtaacagagaggactcacagccagcatagggtcgtgctgtaagccctgttgaggcagttggaaatgacagttcggtagtagttaaggtacccttttaaattacagatttaaacatttggaaagcagctgctggcagctaccgtgatgatcctaaacgggtagctaatgcttttgaaatgatgattaaaactcaggaactggataggaaagatatggaatttattatgcacatgttgtttgatagtacagaaaaataaatgattcactagaccacacggacccaagtggaggatcaggtaatggcaggggttttgcttggatgtaatgctggaaaggacaagagtcctttcctgtcctggggaggatttagaggtggttagaccttggggaggag

SEQ ID NO: 6 - DNA, 962 bp, Artificial Sequence
  For cloning using the gRNA2, W chromosome, "Left arm"
tcgggctaacattagacccgttgtgtcttaatcctgccgtcgggtatacatatactaaaagaacctcctttccctcctataaatcggagcgagacaaggcattctttttttattattattttggttgcctgcccatcagatgtaatgaaagttgcacagggtagggctaagaaggtaaaggagttaaattcccccgggaggttagagattccctgtattgtggttgcctgcccattagacgtaacaaaagttgtgaagggtaggactaaggatccaggtaaagaggttagtcccccagggttagagtccctcctcagaagtaaatgtaaaacataaccacggtaattgtcgttgagtgcgcttgtttgattgttaattgtttgtgctgttattgtatgctgattgtttgtgttgttattatacaaagagctcacatgcatcgttaaaatgggcattggatcacctaggggtgagggaattttgaaaaagtcacttttgggctgtgttttaagtcattggaaagaaatagctggatcccctggtggggttgcacagaaggatgatttaagtacgatggatgcctttgaggcaggcactaggaaccagcagcagtggcagatttgtgatcatggaaagaattggtgggagcatacggcaccaggactcagataagatagctagctaaggtgatgaattgtagatggtgtcagataacgaaagaagaaaaacaaatgtaataaagtgttaaatgccaatatgttttttataatgaggcaatatcctgaatggcattagtgtgggatcaatttggcccagatgaccctctgattttaatggtagaaaatgataagagagagagggagaaaggaagagagtgtaaaacgtgttgttcagcatgtagtattggactgagatgcttcaagcgaaacaagaatgagcaggaggaggatttagagatgcta

SEQ ID NO: 7 - DNA, 478 bp, Artificial Sequence
  For cloning using the gRNA2, W chromosome, "Right arm"
gggcctcaaaatcatggaacccaactccctggagtagaagggtcaggtaatgagtccaaaagagggactataggaaccatgccagtaacagagaggactcacagccagcatagggtcgtgctgtaagccctgttgaggcagttggaaatgacagttcggtagtagttaaggtacccttttaaattacagatttaaacatttggaaagcagctgctggcagctaccgtgatgatcctaaacgggtagctaatgcttttgaaatgatgattaaaactcaggaactggataggaaagatatggaatttattatgcacatgttgtttgatagtacagaaaaataaatgattcactagaccacacggacccaagtggaggatcaggtaatggcaggggttttgcttggatgtaatgctggaaaggacaagagtcctttcctgtcctggggaggatttagaggtggttagaccttggggaggag

SEQ ID NO: 8 - DNA, 669 bp, Artificial Sequence
  A "left arm" for the region upstream to the CMV-promoter
aggcaaggcttgaccgacaattgcatgaagtcgggctaacattagacccgttgtgtcttaatcctgccgtcgggtatacatatactaaaagaacctcctttccctcctataaatcggagcgagacaaggcattctttttttattattattttggttgcctgcccatcagatgtaatgaaagttgcacagggtagggctaagaaggtaaaggagttaaattcccccgggaggttagagattccctgtattgtggttgcctgcccattagacgtaacaaaagttgtgaagggtaggactaaggatccaggtaaagaggttagtcccccagggttagagtccctcctcagaagtaaatgtaaaacataaccacggtaattgtcgttgagtgcgcttgtttgattgttaattgtttgtgctgttattgtatgctgattgtttgtgttgttattatacaaagagctcacatgcatcgttaaaatgggcattggatcacctaggggtgagggaattttgaaaaagtcacttttgggctgtgttttaagtcattggaaagaaatagctggatcccctggtggggttgcacagaaggatgatttaagtacgatggatgcctttgaggcaggcactaggaaccagcagcgatgtacgggccagatatacgcgttgaca

SEQ ID NO: 9 - DNA, 911 bp, Artificial Sequence
  A "right arm" for the region downstream the Neomycin-resistance
ttctatcgccttcttgacgagttcttctgacagtggcagatttgtgatcatggaaagaattggtgggagcatacggcaccaggactcagataagatagctagctaaggtgatgaattgtagatggtgtcagataacgaaagaagaaaaacaaatgtaataaagtgttaaatgccaatatgttttttataatgaggcaatatcctgaatggcattagtgtgggatcaatttggcccagatgaccctctgattttaatggtagaaaatgataagagagagagggagaaaggaagagagtgtaaaacgtgttgttcagcatgtagtattggactgagatgcttcaagcgaaacaagaatgagcaggaggaggatttagagatgctagtagccccaagagggctagggggcctcaaaatcatggaacccaactccctggagtagaagggtcaggtaatgagtccaaaagagggactataggaaccatgccagtaacagagaggactcacagccagcatagggtcgtgctgtaagccctgttgaggcagttggaaatgacagttcggtagtagttaaggtacccttttaaattacagatttaaacatttggaaagcagctgctggcagctaccgtgatgatcctaaacgggtagctaatgcttttgaaatgatgattaaaactcaggaactggataggaaagatatggaatttattatgcacatgttgtttgatagtacagaaaaataaatgattcactagaccacacggacccaagtggaggatcaggtaatggcaggggttttgcttggatgtaatgctggaaaggacaagagtcctttcctgtcctggggaggatttagaggtggttagaccttggggaggagggttcgaaatgaccgaccaagcgacgccca

SEQ ID NO: 10 - DNA, 911 bp, Artificial Sequence
  A "right arm" for the region downstream the polyA site
atctgtgtgttggttttttgtgtgtctagacagtggcagatttgtgatcatggaaagaattggtgggagcatacggcaccaggactcagataagatagctagctaaggtgatgaattgtagatggtgtcagataacgaaagaagaaaaacaaatgtaataaagtgttaaatgccaatatgttttttataatgaggcaatatcctgaatggcattagtgtgggatcaatttggcccagatgaccctctgattttaatggtagaaaatgataagagagagagggagaaaggaagagagtgtaaaacgtgttgttcagcatgtagtattggactgagatgcttcaagcgaaacaagaatgagcaggaggaggatttagagatgctagtagccccaagagggctagggggcctcaaaatcatggaacccaactccctggagtagaagggtcaggtaatgagtccaaaagagggactataggaaccatgccagtaacagagaggactcacagccagcatagggtcgtgctgtaagccctgttgaggcagttggaaatgacagttcggtagtagttaaggtacccttttaaattacagatttaaacatttggaaagcagctgctggcagctaccgtgatgatcctaaacgggtagctaatgcttttgaaatgatgattaaaactcaggaactggataggaaagatatggaatttattatgcacatgttgtttgatagtacagaaaaataaatgattcactagaccacacggacccaagtggaggatcaggtaatggcaggggttttgcttggatgtaatgctggaaaggacaagagtcctttcctgtcctggggaggatttagaggtggttagaccttggggaggagcaagtaagatgcttttctgtgctgcaatag

SEQ ID NO: 11 - DNA, 17 bp, Artificial Sequence
  Guide 3 for Z chromosome
acagacctatgatatgt

SEQ ID NO: 12 - DNA, 17 bp, Artificial Sequence
  Guide 4 for Z chromosome
cgattatcactcacaag

SEQ ID NO: 13 - DNA, 17 bp, Artificial Sequence
  Guide 5 for Z chromosome
ctggttagcatggggac

SEQ ID NO: 14 - DNA, 17 bp, Artificial Sequence
  Guide 6 for Z chromosome
gtaaagagtcagataca

SEQ ID NO: 15 - DNA, 4980 bp, Artificial Sequence
  ENSGALG00000025945_ENSGALG00000023622|chrZ:9156874-9161874
cctgcaggacatgtggacactctgccaggtactgggggaggatcccctccactgctccctgggagatggcaaacatctagagagggacactgcagggatgctgcatgaacacctccagccttctgcaggctgtgatggggtcagggctgaaggtcaacacaagcaatgactgcttgctgacaatgtgggcattgccgaccacagacctatgatatgtgagtggtgagtggggccaggagagcaggacaggagtgtggactcggaggcgcgggcagaggaggtagctcagagcatgagatatattcgccaggtgtcagtggacttctggcagtgcatactgcagagagctttggttgctggccatctggatgatgacaaaatctcagccacagaccatgtgggttggaagagtcctcaggagatcacctttccacctcctgctaaagcacattccctacagtatgtttcacatgacaccgtgctggcagatttttaatatcatcagagaatgacactccatatcctctctgggcagcctttttcagtgctctgtcacccacaaagtaaagtatttgctcatgttctaatggaacttcctatgttctagtttgtgaccattgaaccttgttctgtcactggacagtgctgaaggagcctggccctatccacttgactcccacactttacatatttacaagcatcgataagacccccctcagtcttctccagactagatagccccaggtctcccaaccattccttttatgggagatgcttcaggcccctcatcacctctgtggccctctgctggactgcctgcagtagttccaggtttttttttttgaactggggagcccagaacttgacacggtattccagatgtggcctcaccagcgcagaggagaggggaaggctcacctccctcgacctggtggccatgttttttttaacagacctcaggataccactggccttcttggcccaagggcacactgctggctcatggcccatgggttggcttccaggactctcaggtccttctccgtagagctcctctcaagcaggacaaccctcagcctgtactgatgtgtgcggtgcggttattcctccccacgtgcaagactctacatctgccattgttaaatctcataagcttcctctctgcccaactctccactgtgtacgggccttagtgaatggcagcacagacttctggtgtgaggatagcattcagaacaagctgctgtaccttcccagtcacagaggtgagggtgactggcttgtactttcccagctttgccttcttgcccttttggaagactggagcgacattggccttctggaggaaacggtcctcaggcacccctcctgttctccatgacctttgaaagatgatcgagagcaccttggcagtcacttctgccagctccttcagcacgcatgagtgcatcccgccagtgcccatggatttgtgttcattgaattagcctaggtgacctctgatcagatccttcttgaccaaggggaagacttcctttccccaggttcttatctccagggcctgggattcccaaggggcaatcttagcaggaaaggatgaagtaaaggaggtgtgcagttacagtgctttcatggtgtcctccattactccaatgaggtcacccacctcattcagcagcagacatacattctcccagtcttcctttttctactgccatactaaagtagtccttcatgttgtccttgactgaaggtcacccaacttgatttccagtgagccttagcattccttgtagcattcatgcatgtcctgacaacattcctattttcttcccaagtggccagagaccttttccacactccagaggctttgttcttccattactgcctttccatgagcttcttgctcatctctgcaggtctcatgccacctttgcccgatttcttagtcttagagatgcaccgatcttgaatttggaagaagtggtgcttgaatgacaaccagctctcttggtcccccttgctttccaaagctctaacccatggaatgcctccatgtatgtctgtgaagaggtcaaagtcagctctcctgaagtcgtggttgcaatcctacaaactgcctgatttctcccatgggagatcccgaactccactatctcacagtcactgcactcaaggcttcccccagccttcacatccccagctacaggaagagaagaggctcgaggctacttgcagctgtctgcggaaggcttctccagcttcctcctcttcatcaggcggcctgttgtaaacacccacaacagcgtcacccatcatagcctgtcccttagtcctcacccataaactttctactcattcatcatgcatcccttggcagagctctgtacattccagctgttccctcacataaagagcaactccaccacctcacaccgacgtctgtctgtcctaaaaagtacagagccatccctgagagcattccagtcatgcgagctgccccaccacgtccctctgctgatcgcactgagatcgcggccctacgaccatccatggatctatgactcttcctgtttactccccgcactgtgtgtgatgttacacaggcacttcagagaagaaaagagagcacaggatgccgatttcccttggcaggaccccaggggccgcacgcagcccccacctctatcagcaggtctgagcaggactggagctgcaggcagagcacagctcagccctgagacacctccatgctgcctcctgcacagcctcggccccacagcccccgggaaggagagcacgggtggggtgccgggagccacgctgcgctctgacacactgcgtgtcccctgctcccagcgcgagctgcagggcccgtgcaggaacgagctgggccccaacgtgaccctcggccccggtcactgctgaacgacagcgttcagctctccaggctgcaaagagcgagccgtgaaatggagcaacacgcgggattcccgggtgtgaattcctaaacggattcgaaggtgcccaacaggcagccactgcgtccgcagctgtgcttcggtacctggagacccgcgagcccgtctgttcccaccagcctccagcagccggtgctcgcggatcaaaagaccgccgtgaaggccgcagggccgtccctgggacggagcgccgcccgcttccgccgccagccgcggctccgccctccccgccgagctgacgctggcagcgcgcagagcgcggagcggagccgcggcgctttccggcggcagcgcccgcacggggctcgccgagggccgcgcagagcgctgtgcccggcgggccgcgtcgccgctccggcggcaccgcgattccggcacggagcgcaacgagcgcccgctgcccggctgcaggacgcggtcggggccacaccgcggcggggccgcagcctgccttccgcgggaccgcacgtccggcctccccgaatttggccccgcagcccccgggctgtcaccgtgctgtcaccgtgccgttcacggtttacgggctggttcggcccggttcggcccggttccgtgactggcgggacagagggattcgtggatccgcgcctccgggaagggaaacgggaccccgaataattaaaaacagcggccacgatctgaggggttacaaatgtactaaaacgtactaaaaacaaacagctgcttaacacctcctattccaaaggcccatcgacaccccttggcaccctcaaagtatccccttctgaggtaatgggtaccaagaatgcacggagcccctgggccagtcacagcagggtgcttttgccagtctgtaccggtgaggcctatttcggccacaaacacagtcaattcttgggaacccccattcaccccatgaatataagttgattctgtcccttggtgactcgagggcgtgacagtgcactgtgcaccagggtccaccagggcctcgtattcctgaggttctgatgtgccacaccacgaacccacacggttcaatacactccatcatcctttccccccatggtgggggcagggtccctctatttgttacctctgtcgttcttagagcggttgccatgtcctgcagcaatgggagcgatcacctctttggggattaatcttggtggttaatctgccttgtaattattttacctgtgcttgaaaatgcccctccaggtgaaagcaaactgcagcctgcattctgtggccaaaggaatggaaaagaaggcgttagcaatgccagtggtggcataccacttggcttcttttgactccagttcatactggagttctaacatgtccagaacagcagcgctcagtgggggtgtgacttcattctggccatggtagtctactgtcagcctccattctgcactggctttatgcactggagcacagggcttatggggagcggcggagggagctgggatggttcagtctgcagatgaggaggctcaggggagaccttattgctctctgtaactccatgaagggaggttgtagtgagctgggggtcggtctcttctctcatgtgactagtggtaggactagagggaatggcctccagttgcagcaggggagattcaggctggatgttaggaaatgggctggagtgggctgcccggggaggtggtggagtcaccgaccctggaggtgctcaaggaatgtttagacaccgtgtttagggacatggtatagtgagaactgttggtgatgggtggacagttgggctggatgatcttgtaggtctttttaaagcttggtgattctttgattcgataagtgcaaagtgttgcatttgggtcagagcaatctcacgggtgtgcacaggctgggagaagaactcctgggagaagaagagagcagccctgcagagaaggacttgacatgaaagacttaacgtcagccagactccctctgctctgccctcatgagcctctcctactctgtaaaggtttgggcccccagcaca

SEQ ID NO: 16 - DNA, 4980 bp, Artificial Sequence
  ENSGALG00000015036_ENSGALG00000000438|chrZ:27764943-27769943
aggagtggcttctgaggctggaaacaaggtgctcccctcttgtcaaacagccaattccatctagctccaacccatcctccactggccaaagctgagcccatcgctgatggtgatagcatctgtaatagcatctcagaaaggctaaaagcactgcgcagcagctgagagaaaagagtgagggaaaatgggacagaaacagctctgcagccctcagaggcaatgcagaggagaggcaggaggtgctccaggcatggagcattagtttcttgcagtccaggagttacaggtgatggtgcaggctctgtgcagcccagtgatgactgtttcaggatccatgctgcagcctgtgccagagccaggggataggcttggctgcttagtgcaggacgtggagagcccatgctgagtgcaagctcccaaaaggctaggacagaacaggtgtagtggagtagatcttgtactgtggagcagtcttttcctggaggactaacctgtgaagaggaggactgcgctgaagcggttcatgaagaatgaaaccttgtgggagggaccccacactgaaaaaggagaaaaccacgatgaggaaggagcagcagagagctccccagccctgtgtgcactgccaggagagaaggaagtagaaaacgtgggaatgtgcaggtgtaaagctgagtctgggaaaaaggtgggggtggaataaaggtatttttagtcctatacctttctcatcaacctactttaattgtagattggccataaattaaatgttttccccaggtcaagtctgtttcttgcttgtgatggtggatgatctccctgtcctcatcccaatcctgaagctatttcatcatatattctctccctgccctgtttcaggacagggagtgcaagcagtttggcagccagacgaggttaacccagcaccagaggtttagtcacatgcaagtgagagctattgcctcaacttaaatgggagaaaacattttagcaggttgagtctcaccttgtttatccagattatacagccatgccagcacatgggctgcatgcagcctggcccaacccatcctctagccaccccctgccccatactgaaaatgcagcggctctgccctgccaagctgccaagcctggctccaggcactcacccattgcttacaaacaacaaaacgtcagcgtgtgagcgcgccctgtgagctgcaactggcatggggagggcacagtcagcacaaatacatgacctgcaaattttcacatggaatgtatggagttgcaatcagatactcagctcaaaaaatttaatcatggctccttacctgtcttttttttaacctttctcttagctcagagaggtatacctcacttcacaatcatgccgtattcatgtcattgctttctggcagtacgtacgtttgtgaacagctgttttcaagggtgatgcacaggaagagtaaaatttcattaaaaaatctccaaggagcacatggagagctcactcagaagcctcaccgctgccactgaacaagactgatgcattagtttcatgaaatcaaggctatgtgtcccactggtttcattattttgttactctttctttaaaacaaaaaaattgttttattgcttatatacatcaactatgttgttatatattttccaaaggccgctccaaaagtaatgcctcctgtttcattctgttggcccaccgtgtcagaggcagatggtggtacggcagtagagatggaaccttcccaccaatattccattacatgttgccatgtgatagacagcagcagatgggcactctgacagaatggtatctgacatggaagcgtggatggagcaaagttgtgtcactgaattcctccataaggaaatgagcacccactaacattcactgatgcttgctgaacatttctggagaccaaacagtggatgtgagcacagtgaggtggtgggtggtgcatttcagcagtggtgacaatgacgttgggtcacctctgctggtgcaggttttgatgagtgcagcctgtgaggtcttgttcatcaatggagaaaatgcacaactaatggtggtgactgctgaaaaatagtgttttgtagctgagaattttctctgtcaaacagtgctaattgtgctctttgtatctgttgtagtttccatgggaataaataggaggcattacttgcagactgacctacatatatgtggccccaggcaagtcaacagctgtacgaaaagtccatgcttcctcattataaacggaggaaaaaaagttgtttacagctgtaatgggattataaaaggcaaatggggatagtacagtggtgagaaccagatctatgaaggaaaagccctaagaaaaagagagtgcacagatactcttaaccatctaataactgtttcctccatcctacagctcagagttaagacttacagaggactctagtacttagtaagatgaatacgagctaatagtggcaaaaataatcccagtgcctcaacactgacctgggaaaaaggggcatgtatagaccttctgatattgtgatgctgtgtttgtacacttattatctacattttcagaaattaggttaaacttcagaaaactgaagatctccagggcttgtagcagaccctgaccaccagactggtccccgattatcactcacaagctctcaaaccgattgtggctgtttctcagaggcaactctttgcgctctagcccctctataacatggggcaacttcccctgccccaccttcccttcctgtatcttctgaaaagcttgtagccctcaattgtcacgctccagccatatgaatcatcccaccacgtccctgtgttcacaattaccttctagtcttctaattgcaccatggcttccaattcctcctgtttatcacccacgttgcatccattgatgtagaggcacttcagtcgggctatcagcaatgttaccacctgtgaggagccctcttgagatcttttaggacaatttagaggttttccccactgtttcctaaaattacagcattccctgtcccttcttagtgatatagaactccatccccttccaccatcaaacctagcttaagctctggtaaatgatccagccagtctgcttcccaaaactcttgctcagttgcattctatctgatgcctacatgcccaacaccttcaaggcctgtccaagatcatagaacacaaaggcttgatcatgacaacatccatgcagccaatcattcacatgacccattcctctcctcctttccaggtcccaacggccaactgagagttgtgctctgagctcttcagtgtccttccgagggatgtaaagtcccttttaatgttctgcattttctttgtcacagccttctgagacccaacttgaatgtggaggagtggagagtaatcatcccgctctgattatcagatacattagcctcttcttggcacctctggcagacagaagacttccctggagagattacctggatgataactgggggcctcagtgcctcacagcagcaagtccccagttactaagactctacacctctttggtggcgctagttctgatgtagttcttcagttgcttaacatgcttgttgtttcccaagatttgactgctatctgcaccctccctttcttccagccccagagccttatatcatgagctgagaacattctgtgttcaaaatacaagacacatttatgcaatttcgtattctctacccatatttttgtgatagaaattagggctacttatttcccatagtgatttccatgctgcctaccaggttctaagtcaggtcaccctgccagcttcttccaaaccatgctcaggagtgcatcaaatcacacgcagacccaaggaaaaaatgtaccaaacaatattaccacgcatgcaaactcctcagtagctctgtcccatatgctacaattaggtctgtataggcttgttagatcttgtctacttgattagtgttttccagcaggcctacaatccaacctaaactgaacagacattaaagacatgtttcactaatacaaaacaactccacctagttcaacagtctgctcttttgtgtatggtacctgaaactcttctgttcactgaacttatcccaacatttttcctcctaatgcatactttttctagacgtgatgtgaaagtacagtgttataccctggtgctgcattaatttgcataaccacagcacacaaagcataatcataacacacaaaggcctcctatgaaaacatctgcttaaagtcataggtcacttatttattctccctctagttatgtaccagaatgatgtatgttaataaataatagattattaaatccatcaaaaattagggaagagctctagcacaaaggcaaagcaaagaagctttgaagaagtgcaagtaaaatgaattatttccaaacaactagcttctcactgtcccactaagaacaaagactattcttatgcactgctgtccttaaaattatcagctgctttgtgtttatttcatggagtaacacatgcaatattttttacaagaaataagaaaccacagcagcagaagacgaatctgcttttattgaacgcagaaatagatggacactgaaacaacagaagtttctaccatgttttgctgctgtgagagcaaatctgctgttgatcaactattagttttgaaaagtatatgcaactctgctatcaactccttccccacatcacatctcgtttcaaggagaaccttcctgtccaggcaactagccagggattttaattttaacatttgctatctcagataatcttttaatatttctaggccgtgcacataacccacatagccctaactccagatgttcccagcatcacttagcagtagttccacttgaagcataaatacagcactggcacaacaaatgaagacaattcaagcacgcctttaacaagcatacagaacatacagtttta

SEQ ID NO: 17 - DNA, 4980 bp, Artificial Sequence
  ENSGALG00000012629_ENSGALG00000012628|chrZ:42172748-42177748
acaaattaaatgtattttctcttgatactattttgattataagctattaacttgatttgtaaaagcaccgatattatggttaatgtatgtatggtaactgttgagtcacagcctgaacctctgattgaccacctgcggaaaggtctgggtgagccctgggagcacaggcaaaaacaattcagttgtgcaactggaaggcctctcttagacctcatttaagggctgactgtcactggggaaggatctgattctggagatcccttattggtgaagctttcccctgcaaacctagaatcttctgatgcaagtgagcaatcttcttcccttccctagcagctctctgttgcaccagtccttccatccttgcacctttgttgtaatgcttttcccatggcattgatctgtccagttgctacagtgtagaaacaagaaagtgttttctcaaaacattatacatgcttactatcagatcttacttaacattgataagaagtacacctttcattacaacagtgaacggataggcagcaagcattcagaacaatgaaaaagatctgcgttctattgtaaagcaaacaaaggtgatgacggaacgtttatttgagatacaggcaccatagtacaagatatcaaagaggaattaattcaaccctcccaacaacagttgggaaaaaaaaaggataagctgaggaatgcagccttctccgatttttactctggtgccggaaggaggaggaggagcgggggaaaacccagcggactcagactgcatacgcactctcggaagtacctctgaggcggggtgagaggaagggtggatctaggctccccccgctccacacactcacgtgctcgtgtactggttcaggctgtgacttggcaactcctctacatctatccatctagttagactcaacaagaccatcgtgattcaggagtctgaagatgcttaactctctcagaacgtctagttctcctggcctggtaaatgctatgtttctcatactgcctctctgaagaatgcttcgaatgcttctagtgatgctctaaagttctaaacagaaaaatctggagacagttctggtctttagatagaaaaaatgccaacatgccaaaggatggttacatccttcaagcaaccttgttgcatgctgtacaatagactcatgtaataacttagccgtagtcatcgtatctcttatttacctgttcgttattacattttcctggtactgctttatatttagtcagttgtccttttaagacaaattttttggtgtgtgctaataggcagttaccaaatgttctagagggagggaatataatcagtgagtatgtagatgtatatagatgtataaccagtaagtatacagagaagttagggtggtcttttgagagcatatagctggaaagattatcacatgggaaaaggtaatcagaaataaatggaaaaatgctcaccagtgtcataggctcacaagaaaactccccaaggagcaatctccagtaacagacccttcctcagtggcagtcagcccttaaatggcatctaggagaggtgtagccaggcaccaccccttctgtcacataggtgaattgccttcagctgtgctcctgcagctgactcagtgttcacctcaggtgatcaatcagaggtccagaccatgattcaacatttcccatgcggagggagatgaaacaagactgtcatctcatcttctgaagctgataggagaatggttacaataagtaggtccccttccactggtttagctctgtattactcagtttaaaactttatgtagttaatggagttccatagaatcacatcgctggaaaatgtatgtgatagctatacccaaaaagtgacacagcatcacagcctctaccaggtcctctgcctccagacaggaccttgagctgtgtgatccctttgggatgtttctgtttaagacaggggacacttacacattaggaaactggagtcatgtcggtggaggagaaagtggctgtagaaaaggtaacggacaagaaatccctcactggcttagctgtaaaggtcagaggaaaatcatcttctgttctccatacacatctcctgtaattaggcacctgtgccctttaaaaaagtaaagtaatcaaagagtcatttggtgaaaatagaagccaaacagttacaaaatttagttaatattcaaagacaaaacaactctggttccaaatataaaaccctttgtgtaaacactgcgggaaggtgccaaagagccacctacacaaagagatgccacagagtaatttgcgtaccccaacaataggatcatatatgggcaaaccaaaagaccaacaaagaccccttgcaataatcccttgattggcagaagcaagtgcagcgttagatttagtatgtgtgacaattctgagaataggaaggaatttcactgaaactgtgtgaagatttgtatgttaaatacatataatgagggttatttagctctggggtgtgcatgctatgtggagagatccccatgtgcccagcactgcaatagactaatgtcagctttttaaaccatcatttggtttgaagagtttattatgattttcagaaacagaattatgtattcagtgtctgtacattcttacaagcctgctgttctgtacacatgaaaaagctacttatggtgcaaatcagtatagagaagcagttttgacatacagtggtcatgactgggtgatctgctgtcagaaggtaagacactggtatacagaattgcaaacgtgagatgaagacctcaagtgcaactctgtcatcataccacttctcttgctattatctattcagtgtttgttctaaatattcaggcagaaggcttggtttcacatcaggtgttacatttaagtattctttgcccattttttgctgtttgtatgtgtaacttcagattctcacattgactgtgtagtgtaaatttgcaaatagatgtaacagcttctctttaacatcccatgccaaacttttaatcactttcaatcaatgttggaaatctgcagtacataaattttattttgattcattattcagagaatcagagaaataaggacttttttagaggtttatgtttattttagaaaatataaataaatcttgtatacatagatttccaactagtaaaatttttagctatcgctgtagcatttctatgaggagttttactttttactgtctcttatgaaacttagtggaaacaaagctaggtttcataaaacgtctaatctcatattcatctctctccaaaatatggtgaccttcaaaacaagaacagtttgcttatgtaaacatttcttacattgtattctattacattatcatattcatgaagatactttagaattttgttgctgttagttctgttgtgactggctgcttttctcagcttaagagctctgcagaagtgatgataatatatattctctttgctgagttacaggaatttcctgctttcctctactgtacgttggagcccaggagatcagatccaactaccagaattttatatagctctttgtgatcagtccttccttagttgctgttattcctattgatgcaaacctatttatggtgtattaaatgaagaagatataatgaggacagtctaataatcaaagtttttttctgcagccagtagtacaggtagggtgacatgccttgcataaacagatccagatgaaaggtgtgggtgaggcaataagtcttcaggccctgggctaaggcaggacctgttttgtttcatgagatatgcctaggcctctctatagacagggggagatgtcagagaattctgaagcatcagcagaggctatcttggttttcaggccctgtgctaagtatgagaggaagttgagaacagataatgtgtgcaacaaagttagcaacatgctttttcaaaacagaggaaacgatccataaatactggaacagaacaacctcacagaaatcactgactgtccctttgctggccatggcatcctgaaggttgtgctggtagcactcattgggttgctgtagctgataaggcagtgcaaggacattgggtctgcacctgctatgaacaggcactggggcctccaggagctgctggtattagtcatgggcatcagaggtgaagaaggcacttgtagttctcacagctctggcactgaccgatatttctgctgtagttaatgggattatttgcatgtagtcaacagtttacaggctgatttggctctgctccgcaactagcaggacagagggacccacagatccatgtcctggaaggggataagggaaaaggatagagagatgggcctaaaacaaaacagaagcaacgatctgaggataaacaaagtaatttactaaataagatagtggaatgcatgataacacactatagtacaacataatgcaatgtaattagaactggagctaataaatcaaatataaagagagtgtctgaaagccaaaggccttactctaatgctgtgatgagatggcacccacaaaagagacgagccagatgattgaaagggatgtatggtggtctaccaaggcctgttatctgtttgccctgagcagaaatgatagcagaacagcaaacagtcctctggggaatgtagtagttcttctcttctgggacaggtagctggacctagagcattaactctttaacccccagtacactacatgatgttatgatgtggaataccaataaccaaacatcataaaaccatgacatagtcttatgtcgctgtgttgtaactggaagctgaggatctccactcagtatttctgctgaatgaagcagatctttcagttgaaggagaccaacttaatcatccacttccaaccccttactatggacaggttcaccgttcactagatcaagctgcccagggccccatccaacctagccttgaatgcctccagggatgaggcatccacca

SEQ ID NO: 18 - DNA, 4980 bp, Artificial Sequence
  ENSGALG00000015617_ENSGALG00000027714|chrZ:63363656-63368656
gaaaatctctgccactgattgttttgcagcttagttgtctagttattcgtgagatgttgattcaaacctttgctcagatcaggcacagaagcagtgctgaactttgtttttccgtagccttgctagtgttgtaactgctgtcttagtgaaaacctgcttatttgcatccccttcccaactttgggaaagttgctgtctgtgattccagaattaggactccctcggttgcaacatgactcagattttcagaccttggcttcagaggcacagtggtctttggtgcagagaaaaatgaggctgagaagaccagggccatgatgagtgaggaagatgcaacagaacaagatagagaagagggaagagttttttaggagctccaccagacatactgtagaagcagtgtagatgcacagtaccagtaatgtactccagccaaccactcggtgaagacccatgaaaacctaatgaggttcagtaaggccaagtgcagggtgctgtacttgggtcggggcaatcccaggtatttatacaaactaggggaagatctccttgagagcagccctgcagagaaggacttgggggtcctggtggatgagaagctggacgtgagccagcagtgtgcacctgcagcccggaaggccaactgtgttctgggctgcattaaagaaggggtgaccagcagggagagggaggtgattgtccccctctactcagctcttgtgaggccccatctggagtactgcatccaggcctggagcccccagtacaggaaggacgtggagctcttggagcgggtccagaggaagaccactaagatgatcagagggctggagcacctctcctatgaggaaaggttgagggaactgtccttgtttagcttagagaagagaaggcttcagggaaacctcagtgcagctttccagtacttggaaggagcacataaacaggaaggggaatggctgtttacgagggtggatagtgacaggataagggggaatggttttaaactgagacgggagagttttaggttagatattaggaggaagtttttcacacagagggtggtgacgcactggaacaggttgcccaaggaggttgtggatgccccatccctggaggcattcaaggccaggctggatgtggctctgggcagcctgctctggtggctggcaaccctccacatagcaggggggttgaaactgcgtgatcattgtagtctttttcaacccaggccattctatgattccatgaagactctgtaaggaccccaatgccatcagctgtccccacagcttcagtacccactgccaccacatttttactgagataggtagtttggtagccttcctcccatcttggataggggagggttaactgctggcatttttgttctttcctgcaatatgtgttttctgcatgcattctcttttcacccaaaattttaatgtggacggactttgaggatattctgcatctgcccaatatttcttacagcctcacatctactgatttatgcacagtatcttatatataatgtatattatattatgtatattatgcactgaatcacatctactgtgtatgcacagtaacttctcctatggtactgtaagcccagaaatcccagatatgtcactacaacgtgtctgctatgtattgcttctgtgagacacagatgtgataatcagaggctgtacacagtagaaatgcatacatatcctactgtgaaatctctgaaatctagccttaatcttggaacagaaatgaatatggtgacatcttgatctgatagaattggttgccagtagcacagctgtaatcatccatgatatgaatcaaaccaagcacaggtaaacaggtgagagaaatcatgaacaattacatgcaaacggaccagctaaaatgtgtttgtttgttgttttttttttttcaggtgattcttgattacagtaagatcagaagctgctacattagcagaccagccactgcactcaaggctgtgattcacagcttgcagacctgacagcagttctgtggaagaggcaggtccctgtcaaccagtttaatcaataaatcagtctcgtgtacacaaataatgttatcctgcaccactgctggtgttacactatttcacccaagtttatcaccagcaaactgagtcttatcgttcctactgtgctttgcttttcttgcttagcaaaacatatcagaaaggttttcagttaaaaaaaaaaaaaaaaaaaaaggattatactgcagccatcaaagagttctgttaaagaagttgtggttcatattcttttcaagttctgaagacaatctgacaatagaggagatgagggtttagtggaggtaaatggagctgtttctgaaagtagggcaccgtcgtgaggtaatctcaccactagatgttgctgtaagcatgatgaggggagaagctggagcacaaaaggtgtaaacccaatggttgatcatgcgcactcggacagaggaaatcttcaaaatgggaaagttagctttgaactgatttggtgggttcccattaaaaatgggggacttactgccttattgtctttatgtacccatttgggggatagatgccatacagaaacaccagagcttacggtgtgaattcattgcacatcttattagatcaacaaaatggaataaaagaatacagaagattactactccattgggcatgtggacgttttacaggcctggataaattagatcttaaaaacaaacaaacaaacaaacaaaaaaactccttgcaaagataatgttatgtaatattagttgcaagaagtaagcaaacacacagaactgggagcagaagcaaagcactaagttattaaagcaagttgcacattttgagttgcattttgccactggttttataaacatgtttagcatgtctggtcagaatttgggcaccaggatgcttttaagatgtctgtctatggaacctgtcagtgctcaagaataacttctgttatttggatgctgcaccaaagaattcagaggaagacgagccaagccagacgttatcatagtcactagtaaagtggttctaagcctaattaagacatgtcagaactatgtgttgtgcaaccaaatcctccaaaagagaaatcagaggtgaacttgtgcaataaatatagaagacacgtaaatcctgaggcagttagctaaccatatgaagccaatcatacctgactgctggacgcaggagactgaaccttacagaccctggagaatcactgtttggcctagttaggcctgaatggaatttaccaagattcatgactttaacatggatcaggtgcaaagaaaagaaggctcagttagttcctacaggctaccagatctttttccacctctgctcagcctggagctgtgggctctacctgcccctgaagtgaagtggcatcaactgcaacactttttgcagaggcaaaaatcatcaagtcgtgcctctgcattttaaggtgatggattccaagagatagattccaaacccaacactgagattcctctggtgatgcagatgactgcttactgggatccttctctctctatagcctaatcccatgcagcaccaaaagttgggcacctgaatactatctatcttcctccatctgacctctgctgctggctcatcacgcatggctcctgagcctgacagagccatggggaaagacatggcctgaccttttcagacagcacgacttcctccagtgtgctgcactaacgacaatattaaaaataacactgcaggaaaacatgctgttttctagcaggctggaggaaaaaaaaggtgttcaaggtgagactctataagatcactctttccaaacacagcagttaactcttttctcacttgaagctgaaattcatcttcagtaggtgacggttacaagcagctctccaccggtaagtgaaagtttgctgggtttttttcaggcacttcaagacacgaaggtaattgctgcaacaccttcctagctcttcctgagtactcagcccaaagctacactcttcagggctactctcctagcacggctctctgtaattagcctggctttctaacttatgaattaacgctgcagctactcaacagggcagctttgcagctatgaactttatgcatacactttttattctgggtggtacaaattcattgctaagaaatcttataaactctatggaacacttttaaaagcctacatgtgattaaaaacaaaaaaacaaaaaacactgatatcacatgctatattctctagaaaagagtattttggaaacaattgtaattcacagctcaggagaaagagcaattgttttcctttgtgctggagctggaattctatgcagtataaatacagatgtccaaacaaactcattaaatggtagtcatagcaaatggaggaaaaaaaaagggggggggggggggaactgaagacactgaagaaattctgctgaaattcatggagctgcaacaagaattgatattgattacttcaccatattccgctctaattaactagcacaacactgactgttgtgaaaacaagcatgtgatttgacccaataagtgtttcttttagtaaccaaaaccaaacaacaacaaaccttctggctgaccagatggaggataaattctaacctgatcattctgacacaaatgaggaattatgtaggttggaactgcattccaaagcaaagcatgtttttggcttagttgaacacacagaattcatttttcttgctgattcttgtaactaagggcaggtatgaattggttcccttaaaagaagtccccagaagccatggtcctcaacaagtcttctcagattagcaaggatgaacgactgagaaatcaaaacccaaattcagatctaagagccttcaacagatttgctaaatgaaactagcaaatactgtagaagttaacttgattttgaaataaaacaggatttc

SEQ ID NO: 19 - DNA, 4980 bp, Artificial Sequence
  ENSGALG00000008188_ENSGALG00000008197|chrZ:78777477-78782477
aaaggagtttcttgcctgaaaccccttaagattttgtgtattgttgttgccctggtttcagctgggacaggactgatatccttcacagtatctggtatgatgctgtgttttggttttaggagaaaaccagtgctgatggcacaccgaggttgtagttgcgactgagcagtgctgcacagagccaaggatgtttcagctgcccacactggccttcctctaagggggtgtgagggcacatggagctggagggaaccaaaggggtattccacaccatatgtcactgagcaaagacattgctgcccaggcagagaatacagtggtagaaatacgtcacataggtgcccatctaccccagaactgggccagcgaagaacatcagaacaacaagcatgcgaatcaggctgctcagattgatgtggctcaggtagatctcaactgtcaactgtcacccataaaatggatgagacaggagcaaggcctgcctgtccaaactgaccttggggccccgggcacagctgctcccgagcaaggagaggcagagaattgtggaggaaaccctcttccacctagctccaagggtgcacgctcaatgcttggatgaagattcaagttctcaatgaagaactgcattcaaagacatctttggaggtgacccagactgcctctgggatgaatccagaacaaacagaatcttcccagcaacacctttgtttatcatacacgttcagaaatgcagtgcctgcctggtatttttttaaactcatcacagaggaatctctgagtggagcagaggagtgtttcctcttgcttttttcttccccctttctgtaagaaatgcatatgccagtttccccctaaatgttttcaaactccaaattgtttcctgctggtgacattctcctctccagcactgcctacaccccagctgcgtctgataggaaaagcacccagtaccatgctggcatggcatggtcagtgacacccactggttagcatggggacaaactgccagagcagagggctgctgaaacgccgagtgccaactgacactgttcagctgacagcctcacgagagtgctgcgagggttaagtgaggcaacaaaatacaagtactcaaaaatagaatggaatggaatggaataacagagggaatggggaacaggctgcagtgagaaggaaacccccgtgcaccgaccaacccgctcccagtagcctggtccctaccttgccccactccagcagctccacgaggtactcgaagtgcccatgtccggccatccccagcatggcacagctgtcacctgggagcagcgggggtccggcaggcatcgccggcacccacagcctgggctgggctgaggatgggcttggtgggcagctgggtgctgccgtggcagctgagtgccgtcgtgcaggtgggctcggtgctctctgcagcccacggctcgggacccgtggtgggcatactgctgggcaaggggacggctcggatgtgcatcccagagcagggtgcatgatgtgtgcgcagcggcacacagcagcgcacttgtccccgaggcaccacccggtctgatgaaattccaggttttgtttaagatgaaaatgcatgtgggcatacatttgcacatgagaacacctgctaatgaaacacacagagttgtatgtgcagtctccctggctggtggcatgtctgtgggggcagttaggcaggaagaaaagctccaccatctgtttctgtgtcccgggcttggtgctgccactagagatgggatgcacacagcatgcctgcgtgctgccgaggcagctcagtacctgctgctgggggagagcagccctcagggagctgctgcaaagaccccgtgggatggctggtgaacagtgctggagacatggcagatgtcgcacccctgctccacaccaccctccgctgcagctgcctgcacgatgccatttcagcgtgccacggcttgtttcttcctcttgcagtctcaggttgccgcagcagcagctgcctgaggtctggtggcaaagggcagagcacccagcccactgctctccatgagtgagcgggtagggggcacgccgtgcttcgcttctggtatcgggtggcctgtggagcacatcacccctggacagtgaaaacatgtcaaagggtgttttataacagtatagcatatccctttgaggctgaatttcctgagcttatggatatggtagtaatgctataccaggctctctctgcaggttgctcactgaaacaatataccctttctttctcaagaaatgggactcatgaatagctaccaggcctttctgctactagatactgtagaattacatatatcagatggctcattaatcacatagcttgttattgggacagaggcaggttttcagcatttcccacactgcttttctgcaaatggattaggagtaaagagtcagatacacaggggaccatcactcacttcctaggccatgcttcgtagtttaactccatgcaaggtattttcttgctctgatctaactctagatcactaaatggcacttgtgcaggacacttttccactgtcattttggggggtagaagtgtggtcagagccagggaggcttgcagggcccacaccagctgtggcccaagcagctgctgtacaatggctgtatggcagtatcgatgtgaacttcctgataataaacagaactcagcagcaaataaacccagattgttctgatcagtaacgagaggctgtgcaaaaagctgagaaatgtacagcccttcctgctcaccactacagcccttcatgcagcggcctgctgcactagggcctgcttggccagaggcagggctgcagcttgagatacgcagcacccagtaccccagcaggctgccatgtgcttctgtcaggccatgaattgcacaagttggtatagttttatacagtgtcatgcagaagcacaactcttaccttggcacactgatatggaaagcaaagtgtaaaggaactgtatgtttcttggcttgtgagttccattggttctcccaggacagcagtgacagctctagattttctggttgatctcttccatctaagtttttacttctgaatacatctgtgcagcaaagcctgatgcttttttttttccccctcccctgggatcgtgaaatattattttcccatctccataatacagatgatccactcaaacatgcatcctcagtcgcagtcctcagaagggccttttcccaccatacacctacacgctacaccagactttattggtcaccatgccttgagggattctgcctaacacaggcacacaggaagggctgataccagtaattcattgctgaggagagaaggggcacttcttttatagtagagccacagaatcaccaggattggaaaacacctccaagatcatccaatccaaccacccacctaccaccagtatttcccactaaaccatgccccttggtaccacatctaaaagcatcttctgcaccttcacagcttcattgcctttctcaggacgtgctccagggccttggtgtctttcttgtattgagtggcccaaaattgaacacaatactcgaggtgcagcttcaccaaagctgagtgcagaggggtgatcacctctactaggccttgttttaccccttccccctgcatacctagtttaaagccctttcagcgagccctaccagctcctgggctaggatccatttccccctttaagagaggtgaaacccacccgcaggcatcaggccaggcactgagttaaactgctccatcagctaaccaccccaatgccctgatgtcccttctgatagtcctcaggcttctctcagcgacttcatcactgccagcctgagctatccgtaatggataacaaccagagggctgaaccagactagggagtctcctggtaatgtccctaagtaatgaattcatgggggaaatggatctgtgcagatgcactgccatctcacagggctcaactgtcacagacagttgtcacaaaccagagcagcagagagagcagcaaaggagatatcataaatagtggaaaagggtgccagtgtttgttattgactgcttcactgtgtgtttggaaatcacaaagaaaacaacaaaaaaaccccacagaatacacatttccaagcatgcatgcttcaggtaaggactgcggcccgctttaattcccctggaagcgtccagaggcctacacacaaatcaggccacaacaaacaggttccgtgcaagcagtttgtgagttgtatgaaaatagctttcttccataaagcgtggcattgatgggaactgttactagcagatgaaaatctgccatgcacgacacccttaatggttggagtggttcgactgagttttgcattcctcattctgatggatgctggcaaaaccaagatcacccaacacgtaacactgaatatagctcaccaacagcaacgagccacaccagatactgaggcatctccaaggctacgtctggtggaaagaagagacagtctcaccctgcagtgcaaaagcatcagggcttctgcgtaaggtttattgatcccaaagataggcaagttaatattcatcagtttaatagacaggtactcacattactggagatggcatgccaggagagcctctgccaagtgctcactgccagtggcagccggccagtgcacagcttcttggtgctgtggccatctatataacagaaggaagcaattaagcatcacctatcaagataagcaagatcattcaaagagaataagggtacttggttagagctgcagagcacttcctcacgaatgagtttcttccagctacatgcagatgttacaggcagtttgcttgtgttctagggataacacaaacccctcctcatgggctagctgcctgctcaggctgtggtctgtatttttgcacgtgcactgctagcctttacttcacatttccctttact

SEQ ID NO: 20 - DNA, 681 bp, Artificial Sequence
  pDsRed1
atggtgcgctcctccaagaacgtcatcaaggagttcatgcgcttcaaggtgcgcatggagggcaccgtgaacggccacgagttcgagatcgagggcgagggcgagggccgcccctacgagggccacaacaccgtgaagctgaaggtgaccaagggcggccccctgcccttcgcctgggacatcctgtccccccagttccagtacggctccaaggtgtacgtgaagcaccccgccgacatccccgactacaagaagctgtccttccccgagggcttcaagtgggagcgcgtgatgaacttcgaggacggcggcgtggtgaccgtgacccaggactcctccctgcaggacggctgcttcatctacaaggtgaagttcatcggcgtgaacttcccctccgacggccccgtaatgcagaagaagaccatgggctgggaggcctccaccgagcgcctgtacccccgcgacggcgtgctgaagggcgagatccacaaggccctgaagctgaaggacggcggccactacctggtggagttcaagtccatctacatggccaagaagcccgtgcagctgcccggctactactacgtggactccaagctggacatcacctcccacaacgaggactacaccatcgtggagcagtacgagcgcaccgagggccgccaccacctgttcctgtag

SEQ ID NO: 21 - protein, 226 aa, Artificial Sequence
  pDsRed1
MVRSSKNVIKEFMRFKVRMEGTVNGHEFEIEGEGEGRPYEGHNTVKLKVTKGGPLPFAWDILSPQFQYGSKVYVKHPADIPDYKKLSFPEGFKWERVMNFEDGGVVTVTQDSSLQDGCFIYKVKFIGVNFPSDGPVMQKKTMGWEASTERLYPRDGVLKGEIHKALKLKDGGHYLVEFKSIYMAKKPVQLPGYYYVDSKLDITSHNEDYTIVEQYERTEGRHHLFL

SEQ ID NO: 22 - DNA, 876 bp, Discosoma sp
  misc_feature (1)..(876): red fluorescent protein (FP593) GenBank: AF272711.1
agtttcagccagtgacagggtgagctgccaggtattctaacaagatgagttgttccaagaatgtgatcaaggagttcatgaggttcaaggttcgtatggaaggaacggtcaatgggcacgagtttgaaataaaaggcgaaggtgaagggaggccttacgaaggtcactgttccgtaaagcttatggtaaccaagggtggacctttgccatttgcttttgatattttgtcaccacaatttcagtatggaagcaaggtatatgtcaaacaccctgccgacataccagactataaaaagctgtcatttcctgagggatttaaatgggaaagggtcatgaactttgaagacggtggcgtggttactgtatcccaagattccagtttgaaagacggctgtttcatctacgaggtcaagttcattggggtgaactttccttctgatggacctgttatgcagaggaggacacggggctgggaagccagctctgagcgtttgtatcctcgtgatggggtgctgaaaggagacatccatatggctctgaggctggaaggaggcggccattacctcgttgaattcaaaagtatttacatggtaaagaagccttcagtgcagttgccaggctactattatgttgactccaaactggatatgacgagccacaacgaagattacacagtcgttgagcagtatgaaaaaacccagggacgccaccatccgttcattaagcctctgcagtgaactcggctcagtcatggattagcggtaatggccacaaaaggcacgatgatcgttttttaggaatgcagccaaaaattgaaggttatgacagtagaaatacaagcaacaggctttgcttattaaacatgtaattgaaaac

SEQ ID NO: 23 - protein, 230 aa, Discosoma sp
  MISC_FEATURE (1)..(230): red fluorescent protein D. GenBank: AAG16224.1
MSCSKNVIKEFMRFKVRMEGTVNGHEFEIKGEGEGRPYEGHCSVKLMVTKGGPLPFAFDILSPQFQYGSKVYVKHPADIPDYKKLSFPEGFKWERVMNFEDGGVVTVSQDSSLKDGCFIYEVKFIGVNFPSDGPVMQRRTRGWEASSERLYPRDGVLKGDIHMALRLEGGGHYLVEFKSIYMVKKPSVQLPGYYYVDSKLDMTSHNEDYTVVEQYEKTQGRHHPFIKPLQ

SEQ ID NO: 24 - DNA, 4107 bp, Streptococcus pyogenes
  misc_feature (1)..(4107): M1 GAS Cas9  protein id: AAK33936.1
atggataagaaatactcaataggcttagatatcggcacaaatagcgtcggatgggcggtgatcactgatgaatataaggttccgtctaaaaagttcaaggttctgggaaatacagaccgccacagtatcaaaaaaaatcttataggggctcttttatttgacagtggagagacagcggaagcgactcgtctcaaacggacagctcgtagaaggtatacacgtcggaagaatcgtatttgttatctacaggagattttttcaaatgagatggcgaaagtagatgatagtttctttcatcgacttgaagagtcttttttggtggaagaagacaagaagcatgaacgtcatcctatttttggaaatatagtagatgaagttgcttatcatgagaaatatccaactatctatcatctgcgaaaaaaattggtagattctactgataaagcggatttgcgcttaatctatttggccttagcgcatatgattaagtttcgtggtcattttttgattgagggagatttaaatcctgataatagtgatgtggacaaactatttatccagttggtacaaacctacaatcaattatttgaagaaaaccctattaacgcaagtggagtagatgctaaagcgattctttctgcacgattgagtaaatcaagacgattagaaaatctcattgctcagctccccggtgagaagaaaaatggcttatttgggaatctcattgctttgtcattgggtttgacccctaattttaaatcaaattttgatttggcagaagatgctaaattacagctttcaaaagatacttacgatgatgatttagataatttattggcgcaaattggagatcaatatgctgatttgtttttggcagctaagaatttatcagatgctattttactttcagatatcctaagagtaaatactgaaataactaaggctcccctatcagcttcaatgattaaacgctacgatgaacatcatcaagacttgactcttttaaaagctttagttcgacaacaacttccagaaaagtataaagaaatcttttttgatcaatcaaaaaacggatatgcaggttatattgatgggggagctagccaagaagaattttataaatttatcaaaccaattttagaaaaaatggatggtactgaggaattattggtgaaactaaatcgtgaagatttgctgcgcaagcaacggacctttgacaacggctctattccccatcaaattcacttgggtgagctgcatgctattttgagaagacaagaagacttttatccatttttaaaagacaatcgtgagaagattgaaaaaatcttgacttttcgaattccttattatgttggtccattggcgcgtggcaatagtcgttttgcatggatgactcggaagtctgaagaaacaattaccccatggaattttgaagaagttgtcgataaaggtgcttcagctcaatcatttattgaacgcatgacaaactttgataaaaatcttccaaatgaaaaagtactaccaaaacatagtttgctttatgagtattttacggtttataacgaattgacaaaggtcaaatatgttactgaaggaatgcgaaaaccagcatttctttcaggtgaacagaagaaagccattgttgatttactcttcaaaacaaatcgaaaagtaaccgttaagcaattaaaagaagattatttcaaaaaaatagaatgttttgatagtgttgaaatttcaggagttgaagatagatttaatgcttcattaggtacctaccatgatttgctaaaaattattaaagataaagattttttggataatgaagaaaatgaagatatcttagaggatattgttttaacattgaccttatttgaagatagggagatgattgaggaaagacttaaaacatatgctcacctctttgatgataaggtgatgaaacagcttaaacgtcgccgttatactggttggggacgtttgtctcgaaaattgattaatggtattagggataagcaatctggcaaaacaatattagattttttgaaatcagatggttttgccaatcgcaattttatgcagctgatccatgatgatagtttgacatttaaagaagacattcaaaaagcacaagtgtctggacaaggcgatagtttacatgaacatattgcaaatttagctggtagccctgctattaaaaaaggtattttacagactgtaaaagttgttgatgaattggtcaaagtaatggggcggcataagccagaaaatatcgttattgaaatggcacgtgaaaatcagacaactcaaaagggccagaaaaattcgcgagagcgtatgaaacgaatcgaagaaggtatcaaagaattaggaagtcagattcttaaagagcatcctgttgaaaatactcaattgcaaaatgaaaagctctatctctattatctccaaaatggaagagacatgtatgtggaccaagaattagatattaatcgtttaagtgattatgatgtcgatcacattgttccacaaagtttccttaaagacgattcaatagacaataaggtcttaacgcgttctgataaaaatcgtggtaaatcggataacgttccaagtgaagaagtagtcaaaaagatgaaaaactattggagacaacttctaaacgccaagttaatcactcaacgtaagtttgataatttaacgaaagctgaacgtggaggtttgagtgaacttgataaagctggttttatcaaacgccaattggttgaaactcgccaaatcactaagcatgtggcacaaattttggatagtcgcatgaatactaaatacgatgaaaatgataaacttattcgagaggttaaagtgattaccttaaaatctaaattagtttctgacttccgaaaagatttccaattctataaagtacgtgagattaacaattaccatcatgcccatgatgcgtatctaaatgccgtcgttggaactgctttgattaagaaatatccaaaacttgaatcggagtttgtctatggtgattataaagtttatgatgttcgtaaaatgattgctaagtctgagcaagaaataggcaaagcaaccgcaaaatatttcttttactctaatatcatgaacttcttcaaaacagaaattacacttgcaaatggagagattcgcaaacgccctctaatcgaaactaatggggaaactggagaaattgtctgggataaagggcgagattttgccacagtgcgcaaagtattgtccatgccccaagtcaatattgtcaagaaaacagaagtacagacaggcggattctccaaggagtcaattttaccaaaaagaaattcggacaagcttattgctcgtaaaaaagactgggatccaaaaaaatatggtggttttgatagtccaacggtagcttattcagtcctagtggttgctaaggtggaaaaagggaaatcgaagaagttaaaatccgttaaagagttactagggatcacaattatggaaagaagttcctttgaaaaaaatccgattgactttttagaagctaaaggatataaggaagttaaaaaagacttaatcattaaactacctaaatatagtctttttgagttagaaaacggtcgtaaacggatgctggctagtgccggagaattacaaaaaggaaatgagctggctctgccaagcaaatatgtgaattttttatatttagctagtcattatgaaaagttgaagggtagtccagaagataacgaacaaaaacaattgtttgtggagcagcataagcattatttagatgagattattgagcaaatcagtgaattttctaagcgtgttattttagcagatgccaatttagataaagttcttagtgcatataacaaacatagagacaaaccaatacgtgaacaagcagaaaatattattcatttatttacgttgacgaatcttggagctcccgctgcttttaaatattttgatacaacaattgatcgtaaacgatatacgtctacaaaagaagttttagatgccactcttatccatcaatccatcactggtctttatgaaacacgcattgatttgagtcagctaggaggtgactga

SEQ ID NO: 25 - protein, 1368 aa, Streptococcus pyogenes [sequence omitted]

SEQ ID NO: 26 - DNA, 20 bp, Artificial Sequence
  gRNA7 for Z chromosome locus chrZ_42174515_-1
gtaatacagagctaaaccag

SEQ ID NO: 27 - DNA, 20 bp, Artificial Sequence
  gRNA8 for Z chromosome locus chrZ_9157091_1
acagacctatgatatgtgag

SEQ ID NO: 28 - DNA, 20 bp, Artificial Sequence
  gRNA9 for Z chromosome locus chrZ_27767602_-1
gagcttgtgagtgataatcg

SEQ ID NO: 29 - DNA, 20 bp, Artificial Sequence
  gRNA10 for Z chromosome locus chrZ_78779927_1
gtaaagagtcagatacacag

SEQ ID NO: 30 - DNA, 20 bp, Artificial Sequence
  gRNA11 for Z chromosome locus chrZ_63364946_-1
cagtgggtactgaagctgtg

SEQ ID NO: 31 - DNA, 1012 bp, Artificial Sequence
  Left arm for gRNA7 integration to Chromosome Z ZNF367_HABP4_ENSGALG00000012629_ENSGALG00000012628_chrZ_42174515_ -1
gtgaacggataggcagcaagcattcagaacaatgaaaaagatctgcgttctattgtaaagcaaacaaaggtgatgacggaacgtttatttgagatacaggcaccatagtacaagatatcaaagaggaattaattcaaccctcccaacaacagttgggaaaaaaaaaggataagctgaggaatgcagccttctccgatttttactctggtgccggaaggaggaggaggagcgggggaaaacccagcggactcagactgcatacgcactctcggaagtacctctgaggcggggtgagaggaagggtggatctaggctccccccgctccacacactcacgtgctcgtgtactggttcaggctgtgacttggcaactcctctacatctatccatctagttagactcaacaagaccatcgtgattcaggagtctgaagatgcttaactctctcagaacgtctagttctcctggcctggtaaatgctatgtttctcatactgcctctctgaagaatgcttcgaatgcttctagtgatgctctaaagttctaaacagaaaaatctggagacagttctggtctttagatagaaaaaatgccaacatgccaaaggatggttacatccttcaagcaaccttgttgcatgctgtacaatagactcatgtaataacttagccgtagtcatcgtatctcttatttacctgttcgttattacattttcctggtactgctttatatttagtcagttgtccttttaagacaaattttttggtgtgtgctaataggcagttaccaaatgttctagagggagggaatataatcagtgagtatgtagatgtatatagatgtataaccagtaagtatacagagaagttagggtggtcttttgagagcatatagctggaaagattatcacatgggaaaaggtaatcagaaataaatggaaaaatgctcaccagtgtcataggctcacaagaaaactccccaaggagcaatctccagtaacagacccttcctca

SEQ ID NO: 32 - DNA, 1023 bp, Artificial Sequence
  Right arm for gRNA7 integration to Chromosome Z ZNF367_HABP4_ENSGALG00000012629_ENSGALG00000012628_chrZ_42174515_ -1
gtcatgtcggtggaggagaaagtggctgtagaaaaggtaacggacaagaaatccctcactggcttagctgtaaaggtcagaggaaaatcatcttctgttctccatacacatctcctgtaattaggcacctgtgccctttaaaaaagtaaagtaatcaaagagtcatttggtgaaaatagaagccaaacagttacaaaatttagttaatattcaaagacaaaacaactctggttccaaatataaaaccctttgtgtaaacactgcgggaaggtgccaaagagccacctacacaaagagatgccacagagtaatttgcgtaccccaacaataggatcatatatgggcaaaccaaaagaccaacaaagaccccttgcaataatcccttgattggcagaagcaagtgcagcgttagatttagtatgtgtgacaattctgagaataggaaggaatttcactgaaactgtgtgaagatttgtatgttaaatacatataatgagggttatttagctctggggtgtgcatgctatgtggagagatccccatgtgcccagcactgcaatagactaatgtcagctttttaaaccatcatttggtttgaagagtttattatgattttcagaaacagaattatgtattcagtgtctgtacattcttacaagcctgctgttctgtacacatgaaaaagctacttatggtgcaaatcagtatagagaagcagttttgacatacagtggtcatgactgggtgatctgctgtcagaaggtaagacactggtatacagaattgcaaacgtgagatgaagacctcaagtgcaactctgtcatcataccacttctcttgctattatctattcagtgtttgttctaaatattcaggcagaaggcttggtttcacatcaggtgttacatttaagtattctttgcccattttttgctgtttgtatgtgtaacttcagattctcacattgactgtgtagtgtaaatttgcaaatagatgtaacagcttctctttaacatcccatgc

SEQ ID NO: 33 - DNA, 1014 bp, Artificial Sequence
  Left arm for gRNA8 integration to Chromosome Z ENSGALG00000025945_AVD_ENSGALG00000025945_ENSGALG00000023622_chrZ _9157091_1
ctctgcatggtcacaacggccccaacagcctcccatcccgatgtcaccaatcagttcactattactggtgagcaaccagtccagcactgcatccccctggtggggctgtctgttacgtggctcaggaagttatcctcagtgcattccaggtgctcctggatcgcctgtagctcaccgtgctacttttccagcaggtgtcagggtggtagaagtcccccagcaggacgagagcctgcgattgtgacagcttctgtagctggagggagaatgcttcatcaacaggctccgcttgatcagtgtccctgtactgataccacaaggcttcttttgctgctcccatcttaactctcaccccatcgtggtgttatacgtgcataacatcatgcagtgcactaagagttaaagagttaatgctccagttccgtcgattgtcaataattccaggtgtacctttctcagaagagaagaactacaaatcccttaagatcttactgttccattttcattctccattcagaaggaaaggtaaaactgcagtgtgtgctccctagcattagagtaatttctcccttagctcgttgccaccattttgtttttaggcccacctccttaccttttccctacacccctcctgtgtctctgagacgtgggtccatgggtccctcaaccatagtagacacaaactcagatcaaaccaagccagagctttgacaacccctaagctttcagcttactcagggttgctctgcagggactgctcttcacactctattccttccttgatatagagggcaatgtctcctctcctccttccttacctgtccctcctcatctgcctgttgctgtcagtggccacacttcagccatgggaatcatcccaccctgcttttgtgaaggaaactacattatggttctcaggtagcacagtggcttccatcacctcctgtttgcttcccaagctgtgtgtgttggtgtagaggcacttcagctgggcagctgaagaactggacgcac

SEQ ID NO: 34 - DNA, 1032 bp, Artificial Sequence
  Right arm for gRNA8 integration to Chromosome Z ENSGALG00000025945_AVD_ENSGALG00000025945_ENSGALG00000023622_chrZ _9157091_1
cacctttccacctcctgctaaagcacattccctacagtatgtttcacatgacaccgtgctggcagatttttaatatcatcagagaatgacactccatatcctctctgggcagcctttttcagtgctctgtcacccacaaagtaaagtatttgctcatgttctaatggaacttcctatgttctagtttgtgaccattgaaccttgttctgtcactggacagtgctgaaggagcctggccctatccacttgactcccacactttacatatttacaagcatcgataagacccccctcagtcttctccagactagatagccccaggtctcccaaccattccttttatgggagatgcttcaggcccctcatcacctctgtggccctctgctggactgcctgcagtagttccaggtttttttttttgaactggggagcccagaacttgacacggtattccagatgtggcctcaccagcgcagaggagaggggaaggctcacctccctcgacctggtggccatgttttttttaacagacctcaggataccactggccttcttggcccaagggcacactgctggctcatggcccatgggttggcttccaggactctcaggtccttctccgtagagctcctctcaagcaggacaaccctcagcctgtactgatgtgtgcggtgcggttattcctccccacgtgcaagactctacatctgccattgttaaatctcataagcttcctctctgcccaactctccactgtgtacgggccttagtgaatggcagcacagacttctggtgtgaggatagcattcagaacaagctgctgtaccttcccagtcacagaggtgagggtgactggcttgtactttcccagctttgccttcttgcccttttggaagactggagcgacattggccttctggaggaaacggtcctcaggcacccctcctgttctccatgacctttgaaagatgatcgagagcaccttggcagtcacttctgccagctccttcagcacgcatgagtgcatcccgc

SEQ ID NO: 35 - DNA, 1025 bp, Artificial Sequence
  Left arm for gRNA9 integration to Chromosome Z RIC1_ERMP1_ENSGALG00000015036_ENSGALG00000000438_chrZ_27767602_-1
gcagtacgtacgtttgtgaacagctgttttcaagggtgatgcacaggaagagtaaaatttcattaaaaaatctccaaggagcacatggagagctcactcagaagcctcaccgctgccactgaacaagactgatgcattagtttcatgaaatcaaggctatgtgtcccactggtttcattattttgttactctttctttaaaacaaaaaaattgttttattgcttatatacatcaactatgttgttatatattttccaaaggccgctccaaaagtaatgcctcctgtttcattctgttggcccaccgtgtcagaggcagatggtggtacggcagtagagatggaaccttcccaccaatattccattacatgttgccatgtgatagacagcagcagatgggcactctgacagaatggtatctgacatggaagcgtggatggagcaaagttgtgtcactgaattcctccataaggaaatgagcacccactaacattcactgatgcttgctgaacatttctggagaccaaacagtggatgtgagcacagtgaggtggtgggtggtgcatttcagcagtggtgacaatgacgttgggtcacctctgctggtgcaggttttgatgagtgcagcctgtgaggtcttgttcatcaatggagaaaatgcacaactaatggtggtgactgctgaaaaatagtgttttgtagctgagaattttctctgtcaaacagtgctaattgtgctctttgtatctgttgtagtttccatgggaataaataggaggcattacttgcagactgacctacatatatgtggccccaggcaagtcaacagctgtacgaaaagtccatgcttcctcattataaacggaggaaaaaaagttgtttacagctgtaatgggattataaaaggcaaatggggatagtacagtggtgagaaccagatctatgaaggaaaagccctaagaaaaagagagtgcacagatactcttaaccatctaataactgtttcctccatcctacagctcagag

SEQ ID NO: 36 - DNA, 1040 bp, Artificial Sequence
  Right arm for gRNA9 integration to Chromosome Z RIC1_ERMP1_ENSGALG00000015036_ENSGALG00000000438_chrZ_27767602_-1
tggcttccaattcctcctgtttatcacccacgttgcatccattgatgtagaggcacttcagtcgggctatcagcaatgttaccacctgtgaggagccctcttgagatcttttaggacaatttagaggttttccccactgtttcctaaaattacagcattccctgtcccttcttagtgatatagaactccatccccttccaccatcaaacctagcttaagctctggtaaatgatccagccagtctgcttcccaaaactcttgctcagttgcattctatctgatgcctacatgcccaacaccttcaaggcctgtccaagatcatagaacacaaaggcttgatcatgacaacatccatgcagccaatcattcacatgacccattcctctcctcctttccaggtcccaacggccaactgagagttgtgctctgagctcttcagtgtccttccgagggatgtaaagtcccttttaatgttctgcattttctttgtcacagccttctgagacccaacttgaatgtggaggagtggagagtaatcatcccgctctgattatcagatacattagcctcttcttggcacctctggcagacagaagacttccctggagagattacctggatgataactgggggcctcagtgcctcacagcagcaagtccccagttactaagactctacacctctttggtggcgctagttctgatgtagttcttcagttgcttaacatgcttgttgtttcccaagatttgactgctatctgcaccctccctttcttccagccccagagccttatatcatgagctgagaacattctgtgttcaaaatacaagacacatttatgcaatttcgtattctctacccatatttttgtgatagaaattagggctacttatttcccatagtgatttccatgctgcctaccaggttctaagtcaggtcaccctgccagcttcttccaaaccatgctcaggagtgcatcaaatcacacgcagacccaaggaaaaaatgtaccaaacaatattaccacgcatgcaaactcc

SEQ ID NO: 37 - DNA, 1024 bp, Artificial Sequence
  Left arm for gRNA10 integration to Chromosome Z TRIM36_PGGT1B_ENSGALG00000008188_ENSGALG00000008197_chrZ_78779927 _1Chromosome Z
ctaccttgccccactccagcagctccacgaggtactcgaagtgcccatgtccggccatccccagcatggcacagctgtcacctgggagcagcgggggtccggcaggcatcgccggcacccacagcctgggctgggctgaggatgggcttggtgggcagctgggtgctgccgtggcagctgagtgccgtcgtgcaggtgggctcggtgctctctgcagcccacggctcgggacccgtggtgggcatactgctgggcaaggggacggctcggatgtgcatcccagagcagggtgcatgatgtgtgcgcagcggcacacagcagcgcacttgtccccgaggcaccacccggtctgatgaaattccaggttttgtttaagatgaaaatgcatgtgggcatacatttgcacatgagaacacctgctaatgaaacacacagagttgtatgtgcagtctccctggctggtggcatgtctgtgggggcagttaggcaggaagaaaagctccaccatctgtttctgtgtcccgggcttggtgctgccactagagatgggatgcacacagcatgcctgcgtgctgccgaggcagctcagtacctgctgctgggggagagcagccctcagggagctgctgcaaagaccccgtgggatggctggtgaacagtgctggagacatggcagatgtcgcacccctgctccacaccaccctccgctgcagctgcctgcacgatgccatttcagcgtgccacggcttgtttcttcctcttgcagtctcaggttgccgcagcagcagctgcctgaggtctggtggcaaagggcagagcacccagcccactgctctccatgagtgagcgggtagggggcacgccgtgcttcgcttctggtatcgggtggcctgtggagcacatcacccctggacagtgaaaacatgtcaaagggtgttttataacagtatagcatatccctttgaggctgaatttcctgagcttatggatatggtagtaatgctataccaggctctctctgcag

SEQ ID NO: 38 - DNA, 1022 bp, Artificial Sequence
  Right arm for gRNA10 integration to Chromosome Z TRIM36_PGGT1B_ENSGALG00000008188_ENSGALG00000008197_chrZ_78779927 _1Chromosome Z
cagctgctgtacaatggctgtatggcagtatcgatgtgaacttcctgataataaacagaactcagcagcaaataaacccagattgttctgatcagtaacgagaggctgtgcaaaaagctgagaaatgtacagcccttcctgctcaccactacagcccttcatgcagcggcctgctgcactagggcctgcttggccagaggcagggctgcagcttgagatacgcagcacccagtaccccagcaggctgccatgtgcttctgtcaggccatgaattgcacaagttggtatagttttatacagtgtcatgcagaagcacaactcttaccttggcacactgatatggaaagcaaagtgtaaaggaactgtatgtttcttggcttgtgagttccattggttctcccaggacagcagtgacagctctagattttctggttgatctcttccatctaagtttttacttctgaatacatctgtgcagcaaagcctgatgcttttttttttccccctcccctgggatcgtgaaatattattttcccatctccataatacagatgatccactcaaacatgcatcctcagtcgcagtcctcagaagggccttttcccaccatacacctacacgctacaccagactttattggtcaccatgccttgagggattctgcctaacacaggcacacaggaagggctgataccagtaattcattgctgaggagagaaggggcacttcttttatagtagagccacagaatcaccaggattggaaaacacctccaagatcatccaatccaaccacccacctaccaccagtatttcccactaaaccatgccccttggtaccacatctaaaagcatcttctgcaccttcacagcttcattgcctttctcaggacgtgctccagggccttggtgtctttcttgtattgagtggcccaaaattgaacacaatactcgaggtgcagcttcaccaaagctgagtgcagaggggtgatcacctctactaggccttgttttaccccttcc

SEQ ID NO: 39 - DNA, 1003 bp, Artificial Sequence
  Left arm for gRNA11 integration to Chromosome Z RPS23_ATG10_ENSGALG00000015617_ENSGALG00000027714_chrZ_63364946_- 1
gggttgaaactgcgtgatcattgtagtctttttcaacccaggccattctatgattccatgaagactctgtaaggaccccaatgccatcagctgtccccacagcttcagtacccactgccaccacatttttactgagataggtagtttggtagccttcctcccatcttggataggggagggttaactgctggcatttttgttctttcctgcaatatgtgttttctgcatgcattctcttttcacccaaaattttaatgtggacggactttgaggatattctgcatctgcccaatatttcttacagcctcacatctactgatttatgcacagtatcttatatataatgtatattatattatgtatattatgcactgaatcacatctactgtgtatgcacagtaacttctcctatggtactgtaagcccagaaatcccagatatgtcactacaacgtgtctgctatgtattgcttctgtgagacacagatgtgataatcagaggctgtacacagtagaaatgcatacatatcctactgtgaaatctctgaaatctagccttaatcttggaacagaaatgaatatggtgacatcttgatctgatagaattggttgccagtagcacagctgtaatcatccatgatatgaatcaaaccaagcacaggtaaacaggtgagagaaatcatgaacaattacatgcaaacggaccagctaaaatgtgtttgtttgttgttttttttttttcaggtgattcttgattacagtaagatcagaagctgctacattagcagaccagccactgcactcaaggctgtgattcacagcttgcagacctgacagcagttctgtggaagaggcaggtccctgtcaaccagtttaatcaataaatcagtctcgtgtacacaaataatgttatcctgcaccactgctggtgttacactatttcacccaagtttatcaccagcaaactgagtcttatcgttcctactgtgctttgcttttcttgc

SEQ ID NO: 40 - DNA, 1003 bp, Artificial Sequence
  Right arm for gRNA11 integration to Chromosome Z RPS23_ATG10_ENSGALG00000015617_ENSGALG00000027714_chrZ_63364946_- 1
cagaaacaccagagcttacggtgtgaattcattgcacatcttattagatcaacaaaatggaataaaagaatacagaagattactactccattgggcatgtggacgttttacaggcctggataaattagatcttaaaaacaaacaaacaaacaaacaaaaaaactccttgcaaagataatgttatgtaatattagttgcaagaagtaagcaaacacacagaactgggagcagaagcaaagcactaagttattaaagcaagttgcacattttgagttgcattttgccactggttttataaacatgtttagcatgtctggtcagaatttgggcaccaggatgcttttaagatgtctgtctatggaacctgtcagtgctcaagaataacttctgttatttggatgctgcaccaaagaattcagaggaagacgagccaagccagacgttatcatagtcactagtaaagtggttctaagcctaattaagacatgtcagaactatgtgttgtgcaaccaaatcctccaaaagagaaatcagaggtgaacttgtgcaataaatatagaagacacgtaaatcctgaggcagttagctaaccatatgaagccaatcatacctgactgctggacgcaggagactgaaccttacagaccctggagaatcactgtttggcctagttaggcctgaatggaatttaccaagattcatgactttaacatggatcaggtgcaaagaaaagaaggctcagttagttcctacaggctaccagatctttttccacctctgctcagcctggagctgtgggctctacctgcccctgaagtgaagtggcatcaactgcaacactttttgcagaggcaaaaatcatcaagtcgtgcctctgcattttaaggtgatggattccaagagatagattccaaacccaacactgagattcctctggtgatgcagatgactgcttactgggatccttctctctctatagcctaatcccatgcagcaccaaaag

SEQ ID NO: 41 - DNA, 200 bp, Artificial Sequence
  For cloning using the gRNA3, Z chromosome, "Left arm"
cctgcaggacatgtggacactctgccaggtactgggggaggatcccctccactgctccctgggagatggcaaacatctagagagggacactgcagggatgctgcatgaacacctccagccttctgcaggctgtgatggggtcagggctgaaggtcaacacaagcaatgactgcttgctgacaatgtgggcattgccgacc

SEQ ID NO: 42 - DNA, 258 bp, Artificial Sequence
  For cloning using the gRNA3, Z chromosome, "Right arm"
tggtgagtggggccaggagagcaggacaggagtgtggactcggaggcgcgggcagaggaggtagctcagagcatgagatatattcgccaggtgtcagtggacttctggcagtgcatactgcagagagctttggttgctggccatctggatgatgacaaaatctcagccacagaccatgtgggttggaagagtcctcaggagatcacctttccacctcctgctaaagcacattccctacagtatgtttcacatgacacc

SEQ ID NO: 43 - DNA, 436 bp, Artificial Sequence
  For cloning using the gRNA4, Z chromosome, "Left arm"
tcaacagctgtacgaaaagtccatgcttcctcattataaacggaggaaaaaaagttgtttacagctgtaatgggattataaaaggcaaatggggatagtacagtggtgagaaccagatctatgaaggaaaagccctaagaaaaagagagtgcacagatactcttaaccatctaataactgtttcctccatcctacagctcagagttaagacttacagaggactctagtacttagtaagatgaatacgagctaatagtggcaaaaataatcccagtgcctcaacactgacctgggaaaaaggggcatgtatagaccttctgatattgtgatgctgtgtttgtacacttattatctacattttcagaaattaggttaaacttcagaaaactgaagatctccagggcttgtagcagaccctgaccaccagactggtccc

SEQ ID NO: 44 - DNA, 521 bp, Artificial Sequence
  For cloning using the gRNA4, Z chromosome, "Right arm"
tcaaaccgattgtggctgtttctcagaggcaactctttgcgctctagcccctctataacatggggcaacttcccctgccccaccttcccttcctgtatcttctgaaaagcttgtagccctcaattgtcacgctccagccatatgaatcatcccaccacgtccctgtgttcacaattaccttctagtcttctaattgcaccatggcttccaattcctcctgtttatcacccacgttgcatccattgatgtagaggcacttcagtcgggctatcagcaatgttaccacctgtgaggagccctcttgagatcttttaggacaatttagaggttttccccactgtttcctaaaattacagcattccctgtcccttcttagtgatatagaactccatccccttccaccatcaaacctagcttaagctctggtaaatgatccagccagtctgcttcccaaaactcttgctcagttgcattctatctgatgcctacatgcccaacaccttcaaggcctgtccaagatc

SEQ ID NO: 45 - DNA, 505 bp, Artificial Sequence
  For cloning using the gRNA5, Z chromosome, "Left arm"
gcctgtccaaactgaccttggggccccgggcacagctgctcccgagcaaggagaggcagagaattgtggaggaaaccctcttccacctagctccaagggtgcacgctcaatgcttggatgaagattcaagttctcaatgaagaactgcattcaaagacatctttggaggtgacccagactgcctctgggatgaatccagaacaaacagaatcttcccagcaacacctttgtttatcatacacgttcagaaatgcagtgcctgcctggtatttttttaaactcatcacagaggaatctctgagtggagcagaggagtgtttcctcttgcttttttcttccccctttctgtaagaaatgcatatgccagtttccccctaaatgttttcaaactccaaattgtttcctgctggtgacattctcctctccagcactgcctacaccccagctgcgtctgataggaaaagcacccagtaccatgctggcatggcatggtcagtgacaccca

SEQ ID NO: 46 - DNA, 599 bp, Artificial Sequence
  For cloning using the gRNA5, Z chromosome, "Right arm"
ctgccagagcagagggctgctgaaacgccgagtgccaactgacactgttcagctgacagcctcacgagagtgctgcgagggttaagtgaggcaacaaaatacaagtactcaaaaatagaatggaatggaatggaataacagagggaatggggaacaggctgcagtgagaaggaaacccccgtgcaccgaccaacccgctcccagtagcctggtccctaccttgccccactccagcagctccacgaggtactcgaagtgcccatgtccggccatccccagcatggcacagctgtcacctgggagcagcgggggtccggcaggcatcgccggcacccacagcctgggctgggctgaggatgggcttggtgggcagctgggtgctgccgtggcagctgagtgccgtcgtgcaggtgggctcggtgctctctgcagcccacggctcgggacccgtggtgggcatactgctgggcaaggggacggctcggatgtgcatcccagagcagggtgcatgatgtgtgcgcagcggcacacagcagcgcacttgtccccgaggcaccacccggtctgatgaaattccaggttttgtttaagatgaaaat

SEQ ID NO: 47 - DNA, 453 bp, Artificial Sequence
  For cloning using the gRNA6, Z chromosome, "Left arm"
ttgcagtctcaggttgccgcagcagcagctgcctgaggtctggtggcaaagggcagagcacccagcccactgctctccatgagtgagcgggtagggggcacgccgtgcttcgcttctggtatcgggtggcctgtggagcacatcacccctggacagtgaaaacatgtcaaagggtgttttataacagtatagcatatccctttgaggctgaatttcctgagcttatggatatggtagtaatgctataccaggctctctctgcaggttgctcactgaaacaatataccctttctttctcaagaaatgggactcatgaatagctaccaggcctttctgctactagatactgtagaattacatatatcagatggctcattaatcacatagcttgttattgggacagaggcaggttttcagcatttcccacactgcttttctgcaaatggattagga

SEQ ID NO: 48 - DNA, 439 bp, Artificial Sequence
  For cloning using the gRNA6, Z chromosome, "Right arm"
gggaccatcactcacttcctaggccatgcttcgtagtttaactccatgcaaggtattttcttgctctgatctaactctagatcactaaatggcacttgtgcaggacacttttccactgtcattttggggggtagaagtgtggtcagagccagggaggcttgcagggcccacaccagctgtggcccaagcagctgctgtacaatggctgtatggcagtatcgatgtgaacttcctgataataaacagaactcagcagcaaataaacccagattgttctgatcagtaacgagaggctgtgcaaaaagctgagaaatgtacagcccttcctgctcaccactacagcccttcatgcagcggcctgctgcactagggcctgcttggccagaggcagggctgcagcttgagatacgcagcacccagtaccccagcaggctgccat

SEQ ID NO: 49 - DNA, 22 bp, Artificial Sequence
  LEFT PRIMER
ttggtgtgtgctaataggcagt

SEQ ID NO: 50 - DNA, 20 bp, Artificial Sequence
  RIGHT PRIMER
tagtcctcgttgtgggaggt

SEQ ID NO: 51 - DNA, 20 bp, Artificial Sequence
  LEFT PRIMER
gcattgatctgtccagttgc

SEQ ID NO: 52 - DNA, 20 bp, Artificial Sequence
  RIGHT PRIMER
tactgccaaaaccgcatcac

SEQ ID NO: 53 - DNA, 33 bp, Artificial Sequence
  ChZgRNA_FORWARD PRIMER
tgtatgagaccacgtaatacagagctaaaccag

SEQ ID NO: 54 - DNA, 33 bp, Artificial Sequence
  ChZgRNA_Reverse PRIMER
aaacctggtttagctctgtattacgtggtctca

SEQ ID NO: 55 - DNA, 51 bp, Artificial Sequence
  Primer Forward  for cloning of the 'Left arm' of gRNA 7
acggggtcattagttcatagcccatatatggtgaacggataggcagcaagc

SEQ ID NO: 56 - DNA, 52 bp, Artificial Sequence
  Primer Reverse  for cloning of the 'Left arm' of gRNA 7
ggcgggccatttaccgtaagttatgtaacgtgaggaagggtctgttactgga

SEQ ID NO: 57 - DNA, 51 bp, Artificial Sequence
  Primer Forward  for cloning of the 'Right arm' of gRNA 7
ttctatcgccttcttgacgagttcttctgagtcatgtcggtggaggagaaa

SEQ ID NO: 58 - DNA, 53 bp, Artificial Sequence
  Primer Reverse  for cloning of the 'Right arm' of gRNA 7
gtgatggcaggttgggcgtcgcttggtcgggcatgggatgttaaagagaagct

SEQ ID NO: 59 - DNA, 16 bp, Artificial Sequence
  Repetition of 16 nucleotides
cggtaaatggcccgcc

SEQ ID NO: 60 - DNA, 261 bp, Artificial Sequence
  Flanking left arm of Z chromosome
tggagatcccttattggtgaagctttcccctgcaaacctagaatcttctgatgcaagtgagcaatcttcttcccttccctagcagctctctgttgcaccagtccttccatccttgcacctttgttgtaatgcttttcccatggcattgatctgtccagttgctacagtgtagaaacaagaaagtgttttctcaaaacattatacatgcttactatcagatcttacttaacattgataagaagtacacctttcattacaaca

SEQ ID NO: 61 - DNA, 245 bp, Artificial Sequence
  Flanking right arm of Z chromosome
caaacttttaatcactttcaatcaatgttggaaatctgcagtacataaattttattttgattcattattcagagaatcagagaaataaggacttttttagaggtttatgtttattttagaaaatataaataaatcttgtatacatagatttccaactagtaaaatttttagctatcgctgtagcatttctatgaggagttttactttttactgtctcttatgaaacttagtggaaacaaagctag

SEQ ID NO: 62 - DNA, 1014 bp, Artificial Sequence
  Left arm of Z chromosome
gtgaacggataggcagcaagcattcagaacaatgaaaaagatctgcgttctattgtaaagcaaacaaaggtgatgacggaacgtttatttgagatacaggcaccatagtacaagatatcaaagaggaattaattcaaccctcccaacaacagttgggaaaaaaaaaggataagctgaggaatgcagccttctccgatttttactctggtgccggaaggaggaggaggagcgggggaaaacccagcggactcagactgcatacgcactctcggaagtacctctgaggcggggtgagaggaagggtggatctaggctccccccgctccacacactcacgtgctcgtgtactggttcaggctgtgacttggcaactcctctacatctatccatctagttagactcaacaagaccatcgtgattcaggagtctgaagatgcttaactctctcagaacgtctagttctcctggcctggtaaatgctatgtttctcatactgcctctctgaagaatgcttcgaatgcttctagtgatgctctaaagttctaaacagaaaaatctggagacagttctggtctttagatagaaaaaatgccaacatgccaaaggatggttacatccttcaagcaaccttgttgcatgctgtacaatagactcatgtaataacttagccgtagtcatcgtatctcttatttacctgttcgttattacattttcctggtactgctttatatttagtcagttgtccttttaagacaaattttttggtgtgtgctaataggcagttaccaaatgttctagagggagggaatataatcagtgagtatgtagatgtatatagatgtataaccagtaagtatacagagaagttagggtggtcttttgagagcatatagctggaaagattatcacatgggaaaaggtaatcagaaataaatggaaaaatgctcaccagtgtcataggctcacaagaaaactccccaaggagcaatctccagtaacagacccttcctcagt

SEQ ID NO: 63 - DNA, 629 bp, Artificial Sequence
  CMV Enhancer
tggagttccgcgttacataacttacggtaaatggcccgcctggctgaccgcccaacgacccccgcccattgacgtcaataatgacgtatgttcccatagtaacgccaatagggactttccattgacgtcaatgggtggagtatttacggtaaactgcccacttggcagtacatcaagtgtatcatatgccaagtacgccccctattgacgtcaatgacggtaaatggcccgcctggcattatgcccagtacatgaccttatgggactttcctacttggcagtacatctacgtattagtcatcgctattaccatggtgatgcggttttggcagtacatcaatgggcgtggatagcggtttgactcacggggatttccaagtctccaccccattgacgtcaatgggagtttgttttggcaccaaaatcaacgggactttccaaaatgtcgtaacaactccgccccattgacgcaaatgggcggtaggcgtgtacggtgggaggtctatataagcagagctggtttagtgaaccgtcagatccgctagcgctaccggactcagatctcgagctcaagcttcgaattctgcagtcgacggtaccgcgggcccgggatccaccggtcgccacca

SEQ ID NO: 64 - DNA, 714 bp, Artificial Sequence
  dsRED2 reporter gene
tggcctcctccgagaacgtcatcaccgagttcatgcgcttcaaggtgcgcatggagggcaccgtgaacggccacgagttcgagatcgagggcgagggcgagggccgcccctacgagggccacaacaccgtgaagctgaaggtgaccaagggcggccccctgcccttcgcctgggacatcctgtccccccagttccagtacggctccaaggtgtacgtgaagcaccccgccgacatccccgactacaagaagctgtccttccccgagggcttcaagtgggagcgcgtgatgaacttcgaggacggcggcgtggcgaccgtgacccaggactcctccctgcaggacggctgcttcatctacaaggtgaagttcatcggcgtgaacttcccctccgacggccccgtgatgcagaagaagaccatgggctgggaggcctccaccgagcgcctgtacccccgcgacggcgtgctgaagggcgagacccacaaggccctgaagctgaaggacggcggccactacctggtggagttcaagtccatctacatggccaagaagcccgtgcagctgcccggctactactacgtggacgccaagctggacatcacctcccacaacgaggactacaccatcgtggagcagtacgagcgcaccgagggccgccaccacctgttcctgtagcggccgcgactctagatcataatcagccataccacat

SEQ ID NO: 65 - DNA, 1026 bp, Artificial Sequence
  Right arm of Z chromosome
gagtcatgtcggtggaggagaaagtggctgtagaaaaggtaacggacaagaaatccctcactggcttagctgtaaaggtcagaggaaaatcatcttctgttctccatacacatctcctgtaattaggcacctgtgccctttaaaaaagtaaagtaatcaaagagtcatttggtgaaaatagaagccaaacagttacaaaatttagttaatattcaaagacaaaacaactctggttccaaatataaaaccctttgtgtaaacactgcgggaaggtgccaaagagccacctacacaaagagatgccacagagtaatttgcgtaccccaacaataggatcatatatgggcaaaccaaaagaccaacaaagaccccttgcaataatcccttgattggcagaagcaagtgcagcgttagatttagtatgtgtgacaattctgagaataggaaggaatttcactgaaactgtgtgaagatttgtatgttaaatacatataatgagggttatttagctctggggtgtgcatgctatgtggagagatccccatgtgcccagcactgcaatagactaatgtcagctttttaaaccatcatttggtttgaagagtttattatgattttcagaaacagaattatgtattcagtgtctgtacattcttacaagcctgctgttctgtacacatgaaaaagctacttatggtgcaaatcagtatagagaagcagttttgacatacagtggtcatgactgggtgatctgctgtcagaaggtaagacactggtatacagaattgcaaacgtgagatgaagacctcaagtgcaactctgtcatcataccacttctcttgctattatctattcagtgtttgttctaaatattcaggcagaaggcttggtttcacatcaggtgttacatttaagtattctttgcccattttttgctgtttgtatgtgtaacttcagattctcacattgactgtgtagtgtaaatttgcaaatagatgtaacagcttctctttaacatcccatgca

SEQ ID NO: 66 - DNA, 2618 bp, Artificial Sequence
  Right arm of Z chromosome of Figure 15
tggagatcccttattggtgaagctttcccctgcaaacctagaatcttctgatgcaagtgagcaatcttcttcccttccctagcagctctctgttgcaccagtccttccatccttgcacctttgttgtaatgcttttcccatggcattgatctgtccagttgctacagtgtagaaacaagaaagtgttttctcaaaacattatacatgcttactatcagatcttacttaacattgataagaagtacacctttcattacaacagtgaacggataggcagcaagcattcagaacaatgaaaaagatctgcgttctattgtaaagcaaacaaaggtgatgacggaacgtttatttgagatacaggcaccatagtacaagatatcaaagaggaattaattcaaccctcccaacaacagttgggaaaaaaaaaggataagctgaggaatgcagccttctccgatttttactctggtgccggaaggaggaggaggagcgggggaaaacccagcggactcagactgcatacgcactctcggaagtacctctgaggcggggtgagaggaagggtggatctaggctccccccgctccacacactcacgtgctcgtgtactggttcaggctgtgacttggcaactcctctacatctatccatctagttagactcaacaagaccatcgtgattcaggagtctgaagatgcttaactctctcagaacgtctagttctcctggcctggtaaatgctatgtttctcatactgcctctctgaagaatgcttcgaatgcttctagtgatgctctaaagttctaaacagaaaaatctggagacagttctggtctttagatagaaaaaatgccaacatgccaaaggatggttacatccttcaagcaaccttgttgcatgctgtacaatagactcatgtaataacttagccgtagtcatcgtatctcttatttacctgttcgttattacattttcctggtactgctttatatttagtcagttgtccttttaagacaaattttttggtgtgtgctaataggcagttaccaaatgttctagagggagggaatataatcagtgagtatgtagatgtatatagatgtataaccagtaagtatacagagaagttagggtggtcttttgagagcatatagctggaaagattatcacatgggaaaaggtaatcagaaataaatggaaaaatgctcaccagtgtcataggctcacaagaaaactccccaaggagcaatctccagtaacagacccttcctcagttggagttccgcgttacataacttacggtaaatggcccgcctggctgaccgcccaacgacccccgcccattgacgtcaataatgacgtatgttcccatagtaacgccaatagggactttccattgacgtcaatgggtggagtatttacggtaaactgcccacttggcagtacatcaagtgtatcatatgccaagtacgccccctattgacgtcaatgacggtaaatggcccgcctggcattatgcccagtacatgaccttatgggactttcctacttggcagtacatctacgtattagtcatcgctattaccatggtgatgcggttttggcagtacatcaatgggcgtggatagcggtttgactcacggggatttccaagtctccaccccattgacgtcaatgggagtttgttttggcaccaaaatcaacgggactttccaaaatgtcgtaacaactccgccccattgacgcaaatgggcggtaggcgtgtacggtgggaggtctatataagcagagctggtttagtgaaccgtcagatccgctagcgctaccggactcagatctcgagctcaagcttcgaattctgcagtcgacggtaccgcgggcccgggatccaccggtcgccaccatggcctcctccgagaacgtcatcaccgagttcatgcgcttcaaggtgcgcatggagggcaccgtgaacggccacgagttcgagatcgagggcgagggcgagggccgcccctacgagggccacaacaccgtgaagctgaaggtgaccaagggcggccccctgcccttcgcctgggacatcctgtccccccagttccagtacggctccaaggtgtacgtgaagcaccccgccgacatccccgactacaagaagctgtccttccccgagggcttcaagtgggagcgcgtgatgaacttcgaggacggcggcgtggcgaccgtgacccaggactcctccctgcaggacggctgcttcatctacaaggtgaagttcatcggcgtgaacttcccctccgacggccccgtgatgcagaagaagaccatgggctgggaggcctccaccgagcgcctgtacccccgcgacggcgtgctgaagggcgagacccacaaggccctgaagctgaaggacggcggccactacctggtggagttcaagtccatctacatggccaagaagcccgtgcagctgcccggctactactacgtggacgccaagctggacatcacctcccacaacgaggactacaccatcgtggagcagtacgagcgcaccgagggccgccaccacctgttcctgtagcggccgcgactctagatcataatcagccataccacat

SEQ ID NO: 67 - DNA, 1271 bp, Artificial Sequence
  Left arm of Z chromosome of Figure 15
gagtcatgtcggtggaggagaaagtggctgtagaaaaggtaacggacaagaaatccctcactggcttagctgtaaaggtcagaggaaaatcatcttctgttctccatacacatctcctgtaattaggcacctgtgccctttaaaaaagtaaagtaatcaaagagtcatttggtgaaaatagaagccaaacagttacaaaatttagttaatattcaaagacaaaacaactctggttccaaatataaaaccctttgtgtaaacactgcgggaaggtgccaaagagccacctacacaaagagatgccacagagtaatttgcgtaccccaacaataggatcatatatgggcaaaccaaaagaccaacaaagaccccttgcaataatcccttgattggcagaagcaagtgcagcgttagatttagtatgtgtgacaattctgagaataggaaggaatttcactgaaactgtgtgaagatttgtatgttaaatacatataatgagggttatttagctctggggtgtgcatgctatgtggagagatccccatgtgcccagcactgcaatagactaatgtcagctttttaaaccatcatttggtttgaagagtttattatgattttcagaaacagaattatgtattcagtgtctgtacattcttacaagcctgctgttctgtacacatgaaaaagctacttatggtgcaaatcagtatagagaagcagttttgacatacagtggtcatgactgggtgatctgctgtcagaaggtaagacactggtatacagaattgcaaacgtgagatgaagacctcaagtgcaactctgtcatcataccacttctcttgctattatctattcagtgtttgttctaaatattcaggcagaaggcttggtttcacatcaggtgttacatttaagtattctttgcccattttttgctgtttgtatgtgtaacttcagattctcacattgactgtgtagtgtaaatttgcaaatagatgtaacagcttctctttaacatcccatgcacaaacttttaatcactttcaatcaatgttggaaatctgcagtacataaattttattttgattcattattcagagaatcagagaaataaggacttttttagaggtttatgtttattttagaaaatataaataaatcttgtatacatagatttccaactagtaaaatttttagctatcgctgtagcatttctatgaggagttttactttttactgtctcttatgaaacttagtggaaacaaagctag